European Patent Application EP 4 279 515 A1, published November 22, 2023. Title: Fully Human Single-domain Tandem Chimeric Antigen Receptor (CAR) Targeting CD5 and Use Thereof. Applicant: Nanjing IASO Biotherapeutics Co., Ltd. The sequence listing filed with the application follows.

SEQUENCE LISTING (70 sequences)

SEQ ID NO: 1 - DNA, 63 bp, Artificial Sequence
  FHVH1, FHVH2, FHVH3 and FHVH4 CD8α signal peptide nucleic acid sequence
atggccctgcctgtgacagctctgctcctccctctggccctgctgctccatgccgccagaccc

SEQ ID NO: 2 - protein, 21 aa, Artificial Sequence
  FHVH1, FHVH2, FHVH3 and FHVH4 CD8α signal peptide protein sequence
MALPVTALLLPLALLLHAARP

SEQ ID NO: 3 - DNA, 165 bp, Artificial Sequence
  FHVH1, FHVH2, FHVH3 and FHVH4 CD8α hinge region nucleic acid sequence
ttcgtgcccgtgttcctgcccgccaaacctactactacccctgcacctaggcctcccaccccagccccaacaatcgccagccagcctctgtctctgcggcccgaagcctgtagacctgctgccggcggagccgtgcacaccagaggcctggacttcgcctgcgac

SEQ ID NO: 4 - protein, 55 aa, Artificial Sequence
  FHVH1, FHVH2, FHVH3 and FHVH4 CD8α hinge region protein sequence
FVPVFLPAKPTTTPAPRPPTPAPTIASQPLSLRPEACRPAAGGAVHTRGLDFACD

SEQ ID NO: 5 - DNA, 84 bp, Artificial Sequence
  FHVH1, FHVH2, FHVH3 and FHVH4 CD8α transmembrane region nucleic acid sequence
atctacatctgggcccctctggccggcacctgtggcgtgctgctgctgagcctggtgatcaccctgtactgcaaccaccggaac

SEQ ID NO: 6 - protein, 28 aa, Artificial Sequence
  FHVH1, FHVH2, FHVH3 and FHVH4 CD8α transmembrane region protein sequence
IYIWAPLAGTCGVLLLSLVITLYCNHRN

SEQ ID NO: 7 - DNA, 126 bp, Artificial Sequence
  FHVH1, FHVH2, FHVH3 and FHVH4 4-1BB intracellular co-stimulatory domain nucleic acid sequence
aaacggggcagaaagaaactcctgtatatattcaaacaaccatttatgagaccagtacaaactactcaagaggaagatggctgtagctgccgatttccagaagaagaagaaggaggatgtgaactg

SEQ ID NO: 8 - protein, 42 aa, Artificial Sequence
  FHVH1, FHVH2, FHVH3 and FHVH4 4-1BB intracellular co-stimulatory domain protein sequence
KRGRKKLLYIFKQPFMRPVQTTQEEDGCSCRFPEEEEGGCEL

SEQ ID NO: 9 - DNA, 336 bp, Artificial Sequence
  FHVH1, FHVH2, FHVH3 and FHVH4 CD3z intracellular signaling domain nucleic acid sequence
agagtgaagttcagcagatccgccgacgcccctgcctaccagcagggacagaaccagctgtacaacgagctgaacctgggcagacgggaagagtacgacgtgctggacaagcggagaggccgggaccccgagatgggcggaaagcccagacggaagaacccccaggaaggcctgtataacgaactgcagaaagacaagatggccgaggcctacagcgagatcggcatgaagggcgagcggaggcgcggcaagggccacgatggcctgtaccagggcctgagcaccgccaccaaggacacctacgacgccctgcacatgcaggccctgccccccaga

SEQ ID NO: 10 - protein, 112 aa, Artificial Sequence
  FHVH1, FHVH2, FHVH3 and FHVH4 CD3z intracellular signaling domain protein sequence
RVKFSRSADAPAYQQGQNQLYNELNLGRREEYDVLDKRRGRDPEMGGKPRRKNPQEGLYNELQKDKMAEAYSEIGMKGERRRGKGHDGLYQGLSTATKDTYDALHMQALPPR

SEQ ID NO: 11 - DNA, 54 bp, Artificial Sequence
  FHVH1, FHVH2, FHVH3 and FHVH4 cleaving peptide T2A nucleic acid sequence
gagggaaggggcagcttattaacatgtggcgatgtggaagagaaccccggtccc

SEQ ID NO: 12 - protein, 18 aa, Artificial Sequence
  FHVH1, FHVH2, FHVH3 and FHVH4 cleaving peptide T2A protein sequence
EGRGSLLTCGDVEENPGP

SEQ ID NO: 13 - DNA, 66 bp, Artificial Sequence
  FHVH1, FHVH2, FHVH3 and FHVH4 CSF2RA signal nucleic acid sequence
atgctgctgctcgtgacctctttactgttatgtgagctgccccaccccgcttttttactgatccct

SEQ ID NO: 14 - protein, 22 aa, Artificial Sequence
  FHVH1, FHVH2, FHVH3 and FHVH4 CSF2RA signal protein sequence
MLLLVTSLLLCELPHPAFLLIP

SEQ ID NO: 15 - DNA, 1005 bp, Artificial Sequence
  FHVH1, FHVH2, FHVH3 and FHVH4 tEGFR nucleic acid sequence
cgtaaggtgtgtaacggaatcggcattggcgagttcaaggactctttaagcatcaacgccacaaacatcaagcacttcaagaattgtacctccatcagcggcgatttacacattctccccgtggcttttcgtggcgattccttcacccacaccccccctctggacccccaagagctggacattttaaaaaccgtgaaggagatcaccggctttctgctgatccaagcttggcccgagaatcgtaccgacctccacgccttcgagaatttagagattattcgtggaaggaccaagcagcacggccagttctctttagccgtcgtgtctttaaacattaccagcctcggtttaaggtctttaaaggagattagcgacggcgacgtgatcatctccggcaacaagaacctctgctacgccaacaccatcaactggaagaagctgttcggaaccagcggccaaaagaccaagatcatcagcaatcgtggagagaactcttgtaaggccactggtcaagtttgccacgccctctgtagccccgaaggatgttggggccccgagcctagggactgtgttagctgcagaaacgtgagcagaggcagagagtgtgtggacaaatgcaatttactggaaggagagcctagggagttcgtggagaacagcgaatgtatccagtgccaccccgagtgtttacctcaagccatgaacatcacttgtaccggaaggggccccgataactgcatccaatgcgcccactacatcgacggaccccactgcgtgaaaacttgtcccgccggagtgatgggagagaataacactttagtgtggaagtacgccgacgctggccacgtctgccatctgtgccaccccaactgtacctacggctgcactggtcccggtttagagggatgtcctaccaacggccccaagatcccctccatcgccaccggaatggtgggcgctctgttattactgctggtggtggctctgggcatcggtttattcatg

SEQ ID NO: 16 - protein, 335 aa, Artificial Sequence
  FHVH1, FHVH2, FHVH3 and FHVH4 tEGFR protein sequence
RKVCNGIGIGEFKDSLSINATNIKHFKNCTSISGDLHILPVAFRGDSFTHTPPLDPQELDILKTVKEITGFLLIQAWPENRTDLHAFENLEIIRGRTKQHGQFSLAVVSLNITSLGLRSLKEISDGDVIISGNKNLCYANTINWKKLFGTSGQKTKIISNRGENSCKATGQVCHALCSPEGCWGPEPRDCVSCRNVSRGRECVDKCNLLEGEPREFVENSECIQCHPECLPQAMNITCTGRGPDNCIQCAHYIDGPHCVKTCPAGVMGENNTLVWKYADAGHVCHLCHPNCTYGCTGPGLEGCPTNGPKIPSIATGMVGALLLLLVVALGIGLFM

SEQ ID NO: 17 - DNA, 63 bp, Artificial Sequence
  FHVH3VH1, FHVH2VH1 and FHVH4VH1 CD8α signal peptide nucleic acid sequence
atggccctacctgtgacagccctactgttacccctggccctccttctgcatgctgctagacct

SEQ ID NO: 18 - DNA, 249 bp, Artificial Sequence
  FHVH3VH1, FHVH2VH1 and FHVH4VH1 CD8α hinge region nucleic acid sequence
tttgtgcctgtatttctgcctgccaagcccaccacaacacctgcccctagaccacccacccctgcccccaccattgcttctcagccccttagcttaagacctgaagcctgtagacctgctgctgggggggctgtgcacacaagaggcctggactttgcctgtgacatctacatctgggcccccctggctggcacctgtggggtgctgctgctgagcctggtgatcaccctgtactgcaaccacagaaac

SEQ ID NO: 19 - DNA, 126 bp, Artificial Sequence
  FHVH3VH1, FHVH2VH1 and FHVH4VH1 4-1BB intracellular domain nucleic acid sequence
aagagaggcagaaagaagctgctgtacatcttcaagcagcccttcatgagacctgtgcagaccacccaagaggaggatggctgcagctgcagattccctgaggaggaggaggggggctgtgagctg

SEQ ID NO: 20 - DNA, 336 bp, Artificial Sequence
  FHVH3VH1, FHVH2VH1 and FHVH4VH1 CD3z intracellular signaling domain nucleic acid sequence
agagtgaagttcagcagatctgctgatgcccctgcctatcagcaagggcagaatcagctgtacaatgagctgaatctgggcagaagagaggagtatgatgtgctggacaagagaagaggcagagaccctgagatggggggcaagcctagaagaaagaacccccaagagggcctgtataatgagctgcagaaggacaagatggctgaggcctactctgagattggcatgaagggggagagaagaagaggcaagggccatgatggcctgtaccaaggcctgagcacagccaccaaggacacctatgatgccctacacatgcaagctctgcctcctaga

SEQ ID NO: 21 - DNA, 54 bp, Artificial Sequence
  FHVH3VH1, FHVH2VH1 and FHVH4VH1 cleaving peptide T2A nucleic acid sequence
gaaggaaggggcagcctactgacctgtggggatgtggaggagaaccctggcccc

SEQ ID NO: 22 - DNA, 66 bp, Artificial Sequence
  FHVH3VH1, FHVH2VH1 and FHVH4VH1 CSF2RA signal nucleic acid sequence
atgttgctattagtaaccagcctgctgctgtgtgagctgccccaccctgccttcctgttaatccca

SEQ ID NO: 23 - DNA, 1005 bp, Artificial Sequence
  FHVH3VH1, FHVH2VH1 and FHVH4VH1 tEGFR nucleic acid sequence
cgaaaggtatgtaatggcattggcattggggagtttaaggacagcctgagcatcaatgccaccaacatcaagcacttcaagaactgcacaagcatcagtggggacttgcacatcctgcctgtggccttcagaggggacagcttcacccacaccccccccctggacccccaagagctggacatcctgaagacagtgaaggagatcactggcttcttgctgatccaagcctggcctgagaacagaacagacctgcatgcctttgagaacctggagatcatcagaggcagaaccaagcagcatgggcagttcagcctggctgtggtgagcctgaacatcacaagcctgggcctgagaagcttaaaggagatctctgatggggatgtgatcatctctggcaacaagaacctgtgctatgccaacaccatcaactggaagaagctgtttggcacctctgggcagaagaccaagatcatcagcaacagaggggagaactcctgtaaggccactggccaagtgtgtcatgccctatgcagccctgaggggtgctggggccctgagcctagagactgtgtgagctgcagaaatgtgagcagaggcagagagtgtgtggacaagtgcaacctgctggagggggagcctagagagtttgtggagaactctgagtgtattcagtgtcatcctgagtgcctgccccaagccatgaacatcacctgcactggcagaggccctgacaactgcattcagtgtgcccactacattgatggcccccactgtgtgaagacctgccctgctggggtgatgggggagaacaacaccctggtgtggaagtatgctgatgctggccatgtgtgtcacctgtgccatcccaactgcacctatggctgcactggccctggcctggagggctgccccaccaatggtcccaagattcctagcattgccactggcatggtgggggccctgctcctacttctggtggttgccctgggcattggcctgttcatg

SEQ ID NO: 24 - DNA, 45 bp, Artificial Sequence
  FHVH3VH1, FHVH2VH1 and FHVH4VH1 connecting Linker nucleic acid sequence
gggggggggggctctggggggggtggctcaggtggcggtggctct

SEQ ID NO: 25 - protein, 15 aa, Artificial Sequence
  FHVH3VH1, FHVH2VH1 and FHVH4VH1 connecting Linker protein sequence
GGGGSGGGGSGGGGS

SEQ ID NO: 26 - DNA, 2271 bp, Artificial Sequence
  FHVH1 CAR nucleic acid sequence
atggccctgcctgtgacagctctgctcctccctctggccctgctgctccatgccgccagacccgaagttcagctgctggaaagcggtggtggtctggttcagcctggtggtagcctgcgtctgagctgtgcagcaagcggttttacctttagccatagcgccatgggttgggttcgtcaggcacctggtaaaggtctggaatgggttagcagcatctatgcccgcggcggctatacctattatgcagatagcgttaaaggtcgttttaccattagccgtgataacagcaaaaataccctgtacctgcagatgaatagtctgcgtgcagaggataccgcagtgtattattgtgcgcgcggttaccatctggaatacatggtttctcaggatgtttggggtcaaggtactctggtgaccgtctcctcattcgtgcccgtgttcctgcccgccaaacctactactacccctgcacctaggcctcccaccccagccccaacaatcgccagccagcctctgtctctgcggcccgaagcctgtagacctgctgccggcggagccgtgcacaccagaggcctggacttcgcctgcgacatctacatctgggcccctctggccggcacctgtggcgtgctgctgctgagcctggtgatcaccctgtactgcaaccaccggaacaaacggggcagaaagaaactcctgtatatattcaaacaaccatttatgagaccagtacaaactactcaagaggaagatggctgtagctgccgatttccagaagaagaagaaggaggatgtgaactgagagtgaagttcagcagatccgccgacgcccctgcctaccagcagggacagaaccagctgtacaacgagctgaacctgggcagacgggaagagtacgacgtgctggacaagcggagaggccgggaccccgagatgggcggaaagcccagacggaagaacccccaggaaggcctgtataacgaactgcagaaagacaagatggccgaggcctacagcgagatcggcatgaagggcgagcggaggcgcggcaagggccacgatggcctgtaccagggcctgagcaccgccaccaaggacacctacgacgccctgcacatgcaggccctgccccccagaggatccggagagggaaggggcagcttattaacatgtggcgatgtggaagagaaccccggtcccatgctgctgctcgtgacctctttactgttatgtgagctgccccaccccgcttttttactgatccctcgtaaggtgtgtaacggaatcggcattggcgagttcaaggactctttaagcatcaacgccacaaacatcaagcacttcaagaattgtacctccatcagcggcgatttacacattctccccgtggcttttcgtggcgattccttcacccacaccccccctctggacccccaagagctggacattttaaaaaccgtgaaggagatcaccggctttctgctgatccaagcttggcccgagaatcgtaccgacctccacgccttcgagaatttagagattattcgtggaaggaccaagcagcacggccagttctctttagccgtcgtgtctttaaacattaccagcctcggtttaaggtctttaaaggagattagcgacggcgacgtgatcatctccggcaacaagaacctctgctacgccaacaccatcaactggaagaagctgttcggaaccagcggccaaaagaccaagatcatcagcaatcgtggagagaactcttgtaaggccactggtcaagtttgccacgccctctgtagccccgaaggatgttggggccccgagcctagggactgtgttagctgcagaaacgtgagcagaggcagagagtgtgtggacaaatgcaatttactggaaggagagcctagggagttcgtggagaacagcgaatgtatccagtgccaccccgagtgtttacctcaagccatgaacatcacttgtaccggaaggggccccgataactgcatccaatgcgcccactacatcgacggaccccactgcgtgaaaacttgtcccgccggagtgatgggagagaataacactttagtgtggaagtacgccgacgctggccacgtctgccatctgtgccaccccaactgtacctacggctgcactggtcccggtttagagggatgtcctaccaacggccccaagatcccctccatcgccaccggaatggtgggcgctctgttattactgctggtggtggctctgggcatcggtttattcatg

SEQ ID NO: 27 - protein, 757 aa, Artificial Sequence
  FHVH1 CAR protein sequence
MALPVTALLLPLALLLHAARPEVQLLESGGGLVQPGGSLRLSCAASGFTFSHSAMGWVRQAPGKGLEWVSSIYARGGYTYYADSVKGRFTISRDNSKNTLYLQMNSLRAEDTAVYYCARGYHLEYMVSQDVWGQGTLVTVSSFVPVFLPAKPTTTPAPRPPTPAPTIASQPLSLRPEACRPAAGGAVHTRGLDFACDIYIWAPLAGTCGVLLLSLVITLYCNHRNKRGRKKLLYIFKQPFMRPVQTTQEEDGCSCRFPEEEEGGCELRVKFSRSADAPAYQQGQNQLYNELNLGRREEYDVLDKRRGRDPEMGGKPRRKNPQEGLYNELQKDKMAEAYSEIGMKGERRRGKGHDGLYQGLSTATKDTYDALHMQALPPRGSGEGRGSLLTCGDVEENPGPMLLLVTSLLLCELPHPAFLLIPRKVCNGIGIGEFKDSLSINATNIKHFKNCTSISGDLHILPVAFRGDSFTHTPPLDPQELDILKTVKEITGFLLIQAWPENRTDLHAFENLEIIRGRTKQHGQFSLAVVSLNITSLGLRSLKEISDGDVIISGNKNLCYANTINWKKLFGTSGQKTKIISNRGENSCKATGQVCHALCSPEGCWGPEPRDCVSCRNVSRGRECVDKCNLLEGEPREFVENSECIQCHPECLPQAMNITCTGRGPDNCIQCAHYIDGPHCVKTCPAGVMGENNTLVWKYADAGHVCHLCHPNCTYGCTGPGLEGCPTNGPKIPSIATGMVGALLLLLVVALGIGLFM

SEQ ID NO: 28 - DNA, 2262 bp, Artificial Sequence
  FHVH3 CAR nucleic acid sequence
atggccctgcctgtgacagctctgctcctccctctggccctgctgctccatgccgccagaccccaggtgcagctggtgcagtctggggctgaggtgaagaagcctgggtcctcggtgaaggtctcctgcaaggcttctggaggcaccttcagcaactatgctatcagctgggtgcgacaggcccctggacaagggcttgagtggatgggatggatcagcgcctacaatggtgacacaaaatatgcacagaggctccagggcagagtcaccatgaccacagacacatccacgagcacagcctacatggagctgaggaacctaagatctgacgacacggccgtgtattactgtgcgcgctacgaatctatgtctggtcaggatatctggggtcaaggtactctggtgaccgtctcctcattcgtgcccgtgttcctgcccgccaaacctactactacccctgcacctaggcctcccaccccagccccaacaatcgccagccagcctctgtctctgcggcccgaagcctgtagacctgctgccggcggagccgtgcacaccagaggcctggacttcgcctgcgacatctacatctgggcccctctggccggcacctgtggcgtgctgctgctgagcctggtgatcaccctgtactgcaaccaccggaacaaacggggcagaaagaaactcctgtatatattcaaacaaccatttatgagaccagtacaaactactcaagaggaagatggctgtagctgccgatttccagaagaagaagaaggaggatgtgaactgagagtgaagttcagcagatccgccgacgcccctgcctaccagcagggacagaaccagctgtacaacgagctgaacctgggcagacgggaagagtacgacgtgctggacaagcggagaggccgggaccccgagatgggcggaaagcccagacggaagaacccccaggaaggcctgtataacgaactgcagaaagacaagatggccgaggcctacagcgagatcggcatgaagggcgagcggaggcgcggcaagggccacgatggcctgtaccagggcctgagcaccgccaccaaggacacctacgacgccctgcacatgcaggccctgccccccagaggatccggagagggaaggggcagcttattaacatgtggcgatgtggaagagaaccccggtcccatgctgctgctcgtgacctctttactgttatgtgagctgccccaccccgcttttttactgatccctcgtaaggtgtgtaacggaatcggcattggcgagttcaaggactctttaagcatcaacgccacaaacatcaagcacttcaagaattgtacctccatcagcggcgatttacacattctccccgtggcttttcgtggcgattccttcacccacaccccccctctggacccccaagagctggacattttaaaaaccgtgaaggagatcaccggctttctgctgatccaagcttggcccgagaatcgtaccgacctccacgccttcgagaatttagagattattcgtggaaggaccaagcagcacggccagttctctttagccgtcgtgtctttaaacattaccagcctcggtttaaggtctttaaaggagattagcgacggcgacgtgatcatctccggcaacaagaacctctgctacgccaacaccatcaactggaagaagctgttcggaaccagcggccaaaagaccaagatcatcagcaatcgtggagagaactcttgtaaggccactggtcaagtttgccacgccctctgtagccccgaaggatgttggggccccgagcctagggactgtgttagctgcagaaacgtgagcagaggcagagagtgtgtggacaaatgcaatttactggaaggagagcctagggagttcgtggagaacagcgaatgtatccagtgccaccccgagtgtttacctcaagccatgaacatcacttgtaccggaaggggccccgataactgcatccaatgcgcccactacatcgacggaccccactgcgtgaaaacttgtcccgccggagtgatgggagagaataacactttagtgtggaagtacgccgacgctggccacgtctgccatctgtgccaccccaactgtacctacggctgcactggtcccggtttagagggatgtcctaccaacggccccaagatcccctccatcgccaccggaatggtgggcgctctgttattactgctggtggtggctctgggcatcggtttattcatg

SEQ ID NO: 29 - protein, 754 aa, Artificial Sequence
  FHVH3 CAR protein sequence
MALPVTALLLPLALLLHAARPQVQLVQSGAEVKKPGSSVKVSCKASGGTFSNYAISWVRQAPGQGLEWMGWISAYNGDTKYAQRLQGRVTMTTDTSTSTAYMELRNLRSDDTAVYYCARYESMSGQDIWGQGTLVTVSSFVPVFLPAKPTTTPAPRPPTPAPTIASQPLSLRPEACRPAAGGAVHTRGLDFACDIYIWAPLAGTCGVLLLSLVITLYCNHRNKRGRKKLLYIFKQPFMRPVQTTQEEDGCSCRFPEEEEGGCELRVKFSRSADAPAYQQGQNQLYNELNLGRREEYDVLDKRRGRDPEMGGKPRRKNPQEGLYNELQKDKMAEAYSEIGMKGERRRGKGHDGLYQGLSTATKDTYDALHMQALPPRGSGEGRGSLLTCGDVEENPGPMLLLVTSLLLCELPHPAFLLIPRKVCNGIGIGEFKDSLSINATNIKHFKNCTSISGDLHILPVAFRGDSFTHTPPLDPQELDILKTVKEITGFLLIQAWPENRTDLHAFENLEIIRGRTKQHGQFSLAVVSLNITSLGLRSLKEISDGDVIISGNKNLCYANTINWKKLFGTSGQKTKIISNRGENSCKATGQVCHALCSPEGCWGPEPRDCVSCRNVSRGRECVDKCNLLEGEPREFVENSECIQCHPECLPQAMNITCTGRGPDNCIQCAHYIDGPHCVKTCPAGVMGENNTLVWKYADAGHVCHLCHPNCTYGCTGPGLEGCPTNGPKIPSIATGMVGALLLLLVVALGIGLFM

SEQ ID NO: 30 - DNA, 2670 bp, Artificial Sequence
  FHVH3VH1  CAR nucleic acid sequence
atggccctacctgtgacagccctactgttacccctggccctccttctgcatgctgctagacctcaggtgcagctggtgcagtctggggctgaggtgaagaagcctgggtcctcggtgaaggtctcctgcaaggcttctggaggcaccttcagcaactatgctatcagctgggtgcgacaggcccctggacaagggcttgagtggatgggatggatcagcgcctacaatggtgacacaaaatatgcacagaggctccagggcagagtcaccatgaccacagacacatccacgagcacagcctacatggagctgaggaacctaagatctgacgacacggccgtgtattactgtgcgcgctacgaatctatgtctggtcaggatatctggggtcaaggtactctggtgaccgtctcctcagggggggggggctctggggggggtggctcaggtggcggtggctctgaagttcagctgctggaaagcggtggtggtctggttcagcctggtggtagcctgcgtctgagctgtgcagcaagcggttttacctttagccatagcgccatgggttgggttcgtcaggcacctggtaaaggtctggaatgggttagcagcatctatgcccgcggcggctatacctattatgcagatagcgttaaaggtcgttttaccattagccgtgataacagcaaaaataccctgtacctgcagatgaatagtctgcgtgcagaggataccgcagtgtattattgtgcgcgcggttaccatctggaatacatggtttctcaggatgtttggggtcaaggtactctggtgaccgtctcctcatttgtgcctgtatttctgcctgccaagcccaccacaacacctgcccctagaccacccacccctgcccccaccattgcttctcagccccttagcttaagacctgaagcctgtagacctgctgctgggggggctgtgcacacaagaggcctggactttgcctgtgacatctacatctgggcccccctggctggcacctgtggggtgctgctgctgagcctggtgatcaccctgtactgcaaccacagaaacaagagaggcagaaagaagctgctgtacatcttcaagcagcccttcatgagacctgtgcagaccacccaagaggaggatggctgcagctgcagattccctgaggaggaggaggggggctgtgagctgagagtgaagttcagcagatctgctgatgcccctgcctatcagcaagggcagaatcagctgtacaatgagctgaatctgggcagaagagaggagtatgatgtgctggacaagagaagaggcagagaccctgagatggggggcaagcctagaagaaagaacccccaagagggcctgtataatgagctgcagaaggacaagatggctgaggcctactctgagattggcatgaagggggagagaagaagaggcaagggccatgatggcctgtaccaaggcctgagcacagccaccaaggacacctatgatgccctacacatgcaagctctgcctcctagaggctctggggaaggaaggggcagcctactgacctgtggggatgtggaggagaaccctggccccatgttgctattagtaaccagcctgctgctgtgtgagctgccccaccctgccttcctgttaatcccacgaaaggtatgtaatggcattggcattggggagtttaaggacagcctgagcatcaatgccaccaacatcaagcacttcaagaactgcacaagcatcagtggggacttgcacatcctgcctgtggccttcagaggggacagcttcacccacaccccccccctggacccccaagagctggacatcctgaagacagtgaaggagatcactggcttcttgctgatccaagcctggcctgagaacagaacagacctgcatgcctttgagaacctggagatcatcagaggcagaaccaagcagcatgggcagttcagcctggctgtggtgagcctgaacatcacaagcctgggcctgagaagcttaaaggagatctctgatggggatgtgatcatctctggcaacaagaacctgtgctatgccaacaccatcaactggaagaagctgtttggcacctctgggcagaagaccaagatcatcagcaacagaggggagaactcctgtaaggccactggccaagtgtgtcatgccctatgcagccctgaggggtgctggggccctgagcctagagactgtgtgagctgcagaaatgtgagcagaggcagagagtgtgtggacaagtgcaacctgctggagggggagcctagagagtttgtggagaactctgagtgtattcagtgtcatcctgagtgcctgccccaagccatgaacatcacctgcactggcagaggccctgacaactgcattcagtgtgcccactacattgatggcccccactgtgtgaagacctgccctgctggggtgatgggggagaacaacaccctggtgtggaagtatgctgatgctggccatgtgtgtcacctgtgccatcccaactgcacctatggctgcactggccctggcctggagggctgccccaccaatggtcccaagattcctagcattgccactggcatggtgggggccctgctcctacttctggtggttgccctgggcattggcctgttcatg

SEQ ID NO: 31 - protein, 890 aa, Artificial Sequence
  FHVH3VH1  CAR protein sequence
MALPVTALLLPLALLLHAARPQVQLVQSGAEVKKPGSSVKVSCKASGGTFSNYAISWVRQAPGQGLEWMGWISAYNGDTKYAQRLQGRVTMTTDTSTSTAYMELRNLRSDDTAVYYCARYESMSGQDIWGQGTLVTVSSGGGGSGGGGSGGGGSEVQLLESGGGLVQPGGSLRLSCAASGFTFSHSAMGWVRQAPGKGLEWVSSIYARGGYTYYADSVKGRFTISRDNSKNTLYLQMNSLRAEDTAVYYCARGYHLEYMVSQDVWGQGTLVTVSSFVPVFLPAKPTTTPAPRPPTPAPTIASQPLSLRPEACRPAAGGAVHTRGLDFACDIYIWAPLAGTCGVLLLSLVITLYCNHRNKRGRKKLLYIFKQPFMRPVQTTQEEDGCSCRFPEEEEGGCELRVKFSRSADAPAYQQGQNQLYNELNLGRREEYDVLDKRRGRDPEMGGKPRRKNPQEGLYNELQKDKMAEAYSEIGMKGERRRGKGHDGLYQGLSTATKDTYDALHMQALPPRGSGEGRGSLLTCGDVEENPGPMLLLVTSLLLCELPHPAFLLIPRKVCNGIGIGEFKDSLSINATNIKHFKNCTSISGDLHILPVAFRGDSFTHTPPLDPQELDILKTVKEITGFLLIQAWPENRTDLHAFENLEIIRGRTKQHGQFSLAVVSLNITSLGLRSLKEISDGDVIISGNKNLCYANTINWKKLFGTSGQKTKIISNRGENSCKATGQVCHALCSPEGCWGPEPRDCVSCRNVSRGRECVDKCNLLEGEPREFVENSECIQCHPECLPQAMNITCTGRGPDNCIQCAHYIDGPHCVKTCPAGVMGENNTLVWKYADAGHVCHLCHPNCTYGCTGPGLEGCPTNGPKIPSIATGMVGALLLLLVVALGIGLFM

SEQ ID NO: 32 - DNA, 363 bp, Artificial Sequence
  FHVH1 sdAb nucleic acid sequence
gaagttcagctgctggaaagcggtggtggtctggttcagcctggtggtagcctgcgtctgagctgtgcagcaagcggttttacctttagccatagcgccatgggttgggttcgtcaggcacctggtaaaggtctggaatgggttagcagcatctatgcccgcggcggctatacctattatgcagatagcgttaaaggtcgttttaccattagccgtgataacagcaaaaataccctgtacctgcagatgaatagtctgcgtgcagaggataccgcagtgtattattgtgcgcgcggttaccatctggaatacatggtttctcaggatgtttggggtcaaggtactctggtgaccgtctcctca

SEQ ID NO: 33 - protein, 121 aa, Artificial Sequence
  FHVH1 sdAb protein sequence
EVQLLESGGGLVQPGGSLRLSCAASGFTFSHSAMGWVRQAPGKGLEWVSSIYARGGYTYYADSVKGRFTISRDNSKNTLYLQMNSLRAEDTAVYYCARGYHLEYMVSQDVWGQGTLVTVSS

SEQ ID NO: 34 - DNA, 354 bp, Artificial Sequence
  FHVH3 sdAb nucleic acid sequence
caggtgcagctggtgcagtctggggctgaggtgaagaagcctgggtcctcggtgaaggtctcctgcaaggcttctggaggcaccttcagcaactatgctatcagctgggtgcgacaggcccctggacaagggcttgagtggatgggatggatcagcgcctacaatggtgacacaaaatatgcacagaggctccagggcagagtcaccatgaccacagacacatccacgagcacagcctacatggagctgaggaacctaagatctgacgacacggccgtgtattactgtgcgcgctacgaatctatgtctggtcaggatatctggggtcaaggtactctggtgaccgtctcctca

SEQ ID NO: 35 - protein, 118 aa, Artificial Sequence
  FHVH3 sdAb protein sequence
QVQLVQSGAEVKKPGSSVKVSCKASGGTFSNYAISWVRQAPGQGLEWMGWISAYNGDTKYAQRLQGRVTMTTDTSTSTAYMELRNLRSDDTAVYYCARYESMSGQDIWGQGTLVTVSS

SEQ ID NO: 36 - DNA, 762 bp, Artificial Sequence
  FHVH3VH1  sdAb nucleic acid sequence
caggtgcagctggtgcagtctggggctgaggtgaagaagcctgggtcctcggtgaaggtctcctgcaaggcttctggaggcaccttcagcaactatgctatcagctgggtgcgacaggcccctggacaagggcttgagtggatgggatggatcagcgcctacaatggtgacacaaaatatgcacagaggctccagggcagagtcaccatgaccacagacacatccacgagcacagcctacatggagctgaggaacctaagatctgacgacacggccgtgtattactgtgcgcgctacgaatctatgtctggtcaggatatctggggtcaaggtactctggtgaccgtctcctcagggggggggggctctggggggggtggctcaggtggcggtggctctgaagttcagctgctggaaagcggtggtggtctggttcagcctggtggtagcctgcgtctgagctgtgcagcaagcggttttacctttagccatagcgccatgggttgggttcgtcaggcacctggtaaaggtctggaatgggttagcagcatctatgcccgcggcggctatacctattatgcagatagcgttaaaggtcgttttaccattagccgtgataacagcaaaaataccctgtacctgcagatgaatagtctgcgtgcagaggataccgcagtgtattattgtgcgcgcggttaccatctggaatacatggtttctcaggatgtttggggtcaaggtactctggtgaccgtctcctca

SEQ ID NO: 37 - protein, 254 aa, Artificial Sequence
  FHVH3VH1   sdAb protein sequence
QVQLVQSGAEVKKPGSSVKVSCKASGGTFSNYAISWVRQAPGQGLEWMGWISAYNGDTKYAQRLQGRVTMTTDTSTSTAYMELRNLRSDDTAVYYCARYESMSGQDIWGQGTLVTVSSGGGGSGGGGSGGGGSEVQLLESGGGLVQPGGSLRLSCAASGFTFSHSAMGWVRQAPGKGLEWVSSIYARGGYTYYADSVKGRFTISRDNSKNTLYLQMNSLRAEDTAVYYCARGYHLEYMVSQDVWGQGTLVTVSS

SEQ ID NO: 38 - protein, 8 aa, Artificial Sequence
  FHVH1  HCDR1 amino acid sequence
GFTFSHSA

SEQ ID NO: 39 - protein, 8 aa, Artificial Sequence
  FHVH1  HCDR2 amino acid sequence
IYARGGYT

SEQ ID NO: 40 - protein, 14 aa, Artificial Sequence
  FHVH1  HCDR3 amino acid sequence
ARGYHLEYMVSQDV

SEQ ID NO: 41 - protein, 8 aa, Artificial Sequence
  FHVH3  HCDR1 amino acid sequence
GGTFSNYA

SEQ ID NO: 42 - protein, 8 aa, Artificial Sequence
  FHVH3  HCDR2 amino acid sequence
ISAYNGDT

SEQ ID NO: 43 - protein, 11 aa, Artificial Sequence
  FHVH3  HCDR3 amino acid sequence
ARYESMSGQDI

SEQ ID NO: 44 - DNA, 2670 bp, Artificial Sequence
  FHVH1VH3  CAR nucleic acid sequence
atggccctgcctgtgacagctctgctcctccctctggccctgctgctccatgccgccagacccgaagttcagctgctggaaagcggtggtggtctggttcagcctggtggtagcctgcgtctgagctgtgcagcaagcggttttacctttagccatagcgccatgggttgggttcgtcaggcacctggtaaaggtctggaatgggttagcagcatctatgcccgcggcggctatacctattatgcagatagcgttaaaggtcgttttaccattagccgtgataacagcaaaaataccctgtacctgcagatgaatagtctgcgtgcagaggataccgcagtgtattattgtgcgcgcggttaccatctggaatacatggtttctcaggatgtttggggtcaaggtactctggtgaccgtctcctcagggggggggggctctggggggggtggctcaggtggcggtggctctcaggtgcagctggtgcagtctggggctgaggtgaagaagcctgggtcctcggtgaaggtctcctgcaaggcttctggaggcaccttcagcaactatgctatcagctgggtgcgacaggcccctggacaagggcttgagtggatgggatggatcagcgcctacaatggtgacacaaaatatgcacagaggctccagggcagagtcaccatgaccacagacacatccacgagcacagcctacatggagctgaggaacctaagatctgacgacacggccgtgtattactgtgcgcgctacgaatctatgtctggtcaggatatctggggtcaaggtactctggtgaccgtctcctcattcgtgcccgtgttcctgcccgccaaacctactactacccctgcacctaggcctcccaccccagccccaacaatcgccagccagcctctgtctctgcggcccgaagcctgtagacctgctgccggcggagccgtgcacaccagaggcctggacttcgcctgcgacatctacatctgggcccctctggccggcacctgtggcgtgctgctgctgagcctggtgatcaccctgtactgcaaccaccggaacaaacggggcagaaagaaactcctgtatatattcaaacaaccatttatgagaccagtacaaactactcaagaggaagatggctgtagctgccgatttccagaagaagaagaaggaggatgtgaactgagagtgaagttcagcagatccgccgacgcccctgcctaccagcagggacagaaccagctgtacaacgagctgaacctgggcagacgggaagagtacgacgtgctggacaagcggagaggccgggaccccgagatgggcggaaagcccagacggaagaacccccaggaaggcctgtataacgaactgcagaaagacaagatggccgaggcctacagcgagatcggcatgaagggcgagcggaggcgcggcaagggccacgatggcctgtaccagggcctgagcaccgccaccaaggacacctacgacgccctgcacatgcaggccctgccccccagaggatccggagagggaaggggcagcttattaacatgtggcgatgtggaagagaaccccggtcccatgctgctgctcgtgacctctttactgttatgtgagctgccccaccccgcttttttactgatccctcgtaaggtgtgtaacggaatcggcattggcgagttcaaggactctttaagcatcaacgccacaaacatcaagcacttcaagaattgtacctccatcagcggcgatttacacattctccccgtggcttttcgtggcgattccttcacccacaccccccctctggacccccaagagctggacattttaaaaaccgtgaaggagatcaccggctttctgctgatccaagcttggcccgagaatcgtaccgacctccacgccttcgagaatttagagattattcgtggaaggaccaagcagcacggccagttctctttagccgtcgtgtctttaaacattaccagcctcggtttaaggtctttaaaggagattagcgacggcgacgtgatcatctccggcaacaagaacctctgctacgccaacaccatcaactggaagaagctgttcggaaccagcggccaaaagaccaagatcatcagcaatcgtggagagaactcttgtaaggccactggtcaagtttgccacgccctctgtagccccgaaggatgttggggccccgagcctagggactgtgttagctgcagaaacgtgagcagaggcagagagtgtgtggacaaatgcaatttactggaaggagagcctagggagttcgtggagaacagcgaatgtatccagtgccaccccgagtgtttacctcaagccatgaacatcacttgtaccggaaggggccccgataactgcatccaatgcgcccactacatcgacggaccccactgcgtgaaaacttgtcccgccggagtgatgggagagaataacactttagtgtggaagtacgccgacgctggccacgtctgccatctgtgccaccccaactgtacctacggctgcactggtcccggtttagagggatgtcctaccaacggccccaagatcccctccatcgccaccggaatggtgggcgctctgttattactgctggtggtggctctgggcatcggtttattcatg

SEQ ID NO: 45 - protein, 890 aa, Artificial Sequence
  FHVH1VH3  CAR amino acid sequence
MALPVTALLLPLALLLHAARPEVQLLESGGGLVQPGGSLRLSCAASGFTFSHSAMGWVRQAPGKGLEWVSSIYARGGYTYYADSVKGRFTISRDNSKNTLYLQMNSLRAEDTAVYYCARGYHLEYMVSQDVWGQGTLVTVSSGGGGSGGGGSGGGGSQVQLVQSGAEVKKPGSSVKVSCKASGGTFSNYAISWVRQAPGQGLEWMGWISAYNGDTKYAQRLQGRVTMTTDTSTSTAYMELRNLRSDDTAVYYCARYESMSGQDIWGQGTLVTVSSFVPVFLPAKPTTTPAPRPPTPAPTIASQPLSLRPEACRPAAGGAVHTRGLDFACDIYIWAPLAGTCGVLLLSLVITLYCNHRNKRGRKKLLYIFKQPFMRPVQTTQEEDGCSCRFPEEEEGGCELRVKFSRSADAPAYQQGQNQLYNELNLGRREEYDVLDKRRGRDPEMGGKPRRKNPQEGLYNELQKDKMAEAYSEIGMKGERRRGKGHDGLYQGLSTATKDTYDALHMQALPPRGSGEGRGSLLTCGDVEENPGPMLLLVTSLLLCELPHPAFLLIPRKVCNGIGIGEFKDSLSINATNIKHFKNCTSISGDLHILPVAFRGDSFTHTPPLDPQELDILKTVKEITGFLLIQAWPENRTDLHAFENLEIIRGRTKQHGQFSLAVVSLNITSLGLRSLKEISDGDVIISGNKNLCYANTINWKKLFGTSGQKTKIISNRGENSCKATGQVCHALCSPEGCWGPEPRDCVSCRNVSRGRECVDKCNLLEGEPREFVENSECIQCHPECLPQAMNITCTGRGPDNCIQCAHYIDGPHCVKTCPAGVMGENNTLVWKYADAGHVCHLCHPNCTYGCTGPGLEGCPTNGPKIPSIATGMVGALLLLLVVALGIGLFM

SEQ ID NO: 46 - DNA, 762 bp, Artificial Sequence
  FHVH1VH3  sdAb nucleic acid sequence
gaagttcagctgctggaaagcggtggtggtctggttcagcctggtggtagcctgcgtctgagctgtgcagcaagcggttttacctttagccatagcgccatgggttgggttcgtcaggcacctggtaaaggtctggaatgggttagcagcatctatgcccgcggcggctatacctattatgcagatagcgttaaaggtcgttttaccattagccgtgataacagcaaaaataccctgtacctgcagatgaatagtctgcgtgcagaggataccgcagtgtattattgtgcgcgcggttaccatctggaatacatggtttctcaggatgtttggggtcaaggtactctggtgaccgtctcctcagggggggggggctctggggggggtggctcaggtggcggtggctctcaggtgcagctggtgcagtctggggctgaggtgaagaagcctgggtcctcggtgaaggtctcctgcaaggcttctggaggcaccttcagcaactatgctatcagctgggtgcgacaggcccctggacaagggcttgagtggatgggatggatcagcgcctacaatggtgacacaaaatatgcacagaggctccagggcagagtcaccatgaccacagacacatccacgagcacagcctacatggagctgaggaacctaagatctgacgacacggccgtgtattactgtgcgcgctacgaatctatgtctggtcaggatatctggggtcaaggtactctggtgaccgtctcctca

SEQ ID NO: 47 - protein, 254 aa, Artificial Sequence
  FHVH1VH3  sdAb amino acid sequence
EVQLLESGGGLVQPGGSLRLSCAASGFTFSHSAMGWVRQAPGKGLEWVSSIYARGGYTYYADSVKGRFTISRDNSKNTLYLQMNSLRAEDTAVYYCARGYHLEYMVSQDVWGQGTLVTVSSGGGGSGGGGSGGGGSQVQLVQSGAEVKKPGSSVKVSCKASGGTFSNYAISWVRQAPGQGLEWMGWISAYNGDTKYAQRLQGRVTMTTDTSTSTAYMELRNLRSDDTAVYYCARYESMSGQDIWGQGTLVTVSS

SEQ ID NO: 48 - DNA, 2259 bp, Artificial Sequence
  FHVH2 CAR nucleic acid sequence
atggccctgcctgtgacagctctgctcctccctctggccctgctgctccatgccgccagaccccaggtgcagctggtggagtctgggggaggcttggtacagcctggagggtccctgagactctcctgtgcagcctctggattcaccttcagtagttatgaaatgaactgggtccgccaggctccagggaaggggctggagtgggtttcatacattagtagtagtggtagtaccatatactacgcagactctgtgaagggccgattcaccatctccagagacaacgccaagaactcactgtatctgcaaatgaacagtctgagagccgaggacacggctgtttattactgtgcgagagtcgcccagagagaaggggacgtctggggcaaagggaccacggtcaccgtctcctcattcgtgcccgtgttcctgcccgccaaacctactactacccctgcacctaggcctcccaccccagccccaacaatcgccagccagcctctgtctctgcggcccgaagcctgtagacctgctgccggcggagccgtgcacaccagaggcctggacttcgcctgcgacatctacatctgggcccctctggccggcacctgtggcgtgctgctgctgagcctggtgatcaccctgtactgcaaccaccggaacaaacggggcagaaagaaactcctgtatatattcaaacaaccatttatgagaccagtacaaactactcaagaggaagatggctgtagctgccgatttccagaagaagaagaaggaggatgtgaactgagagtgaagttcagcagatccgccgacgcccctgcctaccagcagggacagaaccagctgtacaacgagctgaacctgggcagacgggaagagtacgacgtgctggacaagcggagaggccgggaccccgagatgggcggaaagcccagacggaagaacccccaggaaggcctgtataacgaactgcagaaagacaagatggccgaggcctacagcgagatcggcatgaagggcgagcggaggcgcggcaagggccacgatggcctgtaccagggcctgagcaccgccaccaaggacacctacgacgccctgcacatgcaggccctgccccccagaggatccggagagggaaggggcagcttattaacatgtggcgatgtggaagagaaccccggtcccatgctgctgctcgtgacctctttactgttatgtgagctgccccaccccgcttttttactgatccctcgtaaggtgtgtaacggaatcggcattggcgagttcaaggactctttaagcatcaacgccacaaacatcaagcacttcaagaattgtacctccatcagcggcgatttacacattctccccgtggcttttcgtggcgattccttcacccacaccccccctctggacccccaagagctggacattttaaaaaccgtgaaggagatcaccggctttctgctgatccaagcttggcccgagaatcgtaccgacctccacgccttcgagaatttagagattattcgtggaaggaccaagcagcacggccagttctctttagccgtcgtgtctttaaacattaccagcctcggtttaaggtctttaaaggagattagcgacggcgacgtgatcatctccggcaacaagaacctctgctacgccaacaccatcaactggaagaagctgttcggaaccagcggccaaaagaccaagatcatcagcaatcgtggagagaactcttgtaaggccactggtcaagtttgccacgccctctgtagccccgaaggatgttggggccccgagcctagggactgtgttagctgcagaaacgtgagcagaggcagagagtgtgtggacaaatgcaatttactggaaggagagcctagggagttcgtggagaacagcgaatgtatccagtgccaccccgagtgtttacctcaagccatgaacatcacttgtaccggaaggggccccgataactgcatccaatgcgcccactacatcgacggaccccactgcgtgaaaacttgtcccgccggagtgatgggagagaataacactttagtgtggaagtacgccgacgctggccacgtctgccatctgtgccaccccaactgtacctacggctgcactggtcccggtttagagggatgtcctaccaacggccccaagatcccctccatcgccaccggaatggtgggcgctctgttattactgctggtggtggctctgggcatcggtttattcatg

SEQ ID NO: 49 - protein, 753 aa, Artificial Sequence
  FHVH2 CAR protein sequence
MALPVTALLLPLALLLHAARPQVQLVESGGGLVQPGGSLRLSCAASGFTFSSYEMNWVRQAPGKGLEWVSYISSSGSTIYYADSVKGRFTISRDNAKNSLYLQMNSLRAEDTAVYYCARVAQREGDVWGKGTTVTVSSFVPVFLPAKPTTTPAPRPPTPAPTIASQPLSLRPEACRPAAGGAVHTRGLDFACDIYIWAPLAGTCGVLLLSLVITLYCNHRNKRGRKKLLYIFKQPFMRPVQTTQEEDGCSCRFPEEEEGGCELRVKFSRSADAPAYQQGQNQLYNELNLGRREEYDVLDKRRGRDPEMGGKPRRKNPQEGLYNELQKDKMAEAYSEIGMKGERRRGKGHDGLYQGLSTATKDTYDALHMQALPPRGSGEGRGSLLTCGDVEENPGPMLLLVTSLLLCELPHPAFLLIPRKVCNGIGIGEFKDSLSINATNIKHFKNCTSISGDLHILPVAFRGDSFTHTPPLDPQELDILKTVKEITGFLLIQAWPENRTDLHAFENLEIIRGRTKQHGQFSLAVVSLNITSLGLRSLKEISDGDVIISGNKNLCYANTINWKKLFGTSGQKTKIISNRGENSCKATGQVCHALCSPEGCWGPEPRDCVSCRNVSRGRECVDKCNLLEGEPREFVENSECIQCHPECLPQAMNITCTGRGPDNCIQCAHYIDGPHCVKTCPAGVMGENNTLVWKYADAGHVCHLCHPNCTYGCTGPGLEGCPTNGPKIPSIATGMVGALLLLLVVALGIGLFM

SEQ ID NO: 50 - DNA, 2277 bp, Artificial Sequence
  FHVH4 CAR nucleic acid sequence
atggccctgcctgtgacagctctgctcctccctctggccctgctgctccatgccgccagaccccaggtccagctggtgcagtctggggctgaggtgaaaaagcccggggagtctctgaggatctcctgtaaggcttctggatacagttttagcaaccattggatcggctgggtgcgccagaagcccgggaaaggcctggagtggatggggagcgtctatcctggtgactccgataccagatacagcccgtccttccaaggccacgtcactgtctcagccgacaagtccatgaataccgcctacctgcagtggagcagcctgaagacctcggacaccgccatgtattattgtgcgagaggtgggactattgacggtgactacggggggaggcaagacttctggggccagggaaccatggtcaccgtctcttcattcgtgcccgtgttcctgcccgccaaacctactactacccctgcacctaggcctcccaccccagccccaacaatcgccagccagcctctgtctctgcggcccgaagcctgtagacctgctgccggcggagccgtgcacaccagaggcctggacttcgcctgcgacatctacatctgggcccctctggccggcacctgtggcgtgctgctgctgagcctggtgatcaccctgtactgcaaccaccggaacaaacggggcagaaagaaactcctgtatatattcaaacaaccatttatgagaccagtacaaactactcaagaggaagatggctgtagctgccgatttccagaagaagaagaaggaggatgtgaactgagagtgaagttcagcagatccgccgacgcccctgcctaccagcagggacagaaccagctgtacaacgagctgaacctgggcagacgggaagagtacgacgtgctggacaagcggagaggccgggaccccgagatgggcggaaagcccagacggaagaacccccaggaaggcctgtataacgaactgcagaaagacaagatggccgaggcctacagcgagatcggcatgaagggcgagcggaggcgcggcaagggccacgatggcctgtaccagggcctgagcaccgccaccaaggacacctacgacgccctgcacatgcaggccctgccccccagaggatccggagagggaaggggcagcttattaacatgtggcgatgtggaagagaaccccggtcccatgctgctgctcgtgacctctttactgttatgtgagctgccccaccccgcttttttactgatccctcgtaaggtgtgtaacggaatcggcattggcgagttcaaggactctttaagcatcaacgccacaaacatcaagcacttcaagaattgtacctccatcagcggcgatttacacattctccccgtggcttttcgtggcgattccttcacccacaccccccctctggacccccaagagctggacattttaaaaaccgtgaaggagatcaccggctttctgctgatccaagcttggcccgagaatcgtaccgacctccacgccttcgagaatttagagattattcgtggaaggaccaagcagcacggccagttctctttagccgtcgtgtctttaaacattaccagcctcggtttaaggtctttaaaggagattagcgacggcgacgtgatcatctccggcaacaagaacctctgctacgccaacaccatcaactggaagaagctgttcggaaccagcggccaaaagaccaagatcatcagcaatcgtggagagaactcttgtaaggccactggtcaagtttgccacgccctctgtagccccgaaggatgttggggccccgagcctagggactgtgttagctgcagaaacgtgagcagaggcagagagtgtgtggacaaatgcaatttactggaaggagagcctagggagttcgtggagaacagcgaatgtatccagtgccaccccgagtgtttacctcaagccatgaacatcacttgtaccggaaggggccccgataactgcatccaatgcgcccactacatcgacggaccccactgcgtgaaaacttgtcccgccggagtgatgggagagaataacactttagtgtggaagtacgccgacgctggccacgtctgccatctgtgccaccccaactgtacctacggctgcactggtcccggtttagagggatgtcctaccaacggccccaagatcccctccatcgccaccggaatggtgggcgctctgttattactgctggtggtggctctgggcatcggtttattcatg

SEQ ID NO: 51 - protein, 759 aa, Artificial Sequence
  FHVH4 CAR protein sequence
MALPVTALLLPLALLLHAARPQVQLVQSGAEVKKPGESLRISCKASGYSFSNHWIGWVRQKPGKGLEWMGSVYPGDSDTRYSPSFQGHVTVSADKSMNTAYLQWSSLKTSDTAMYYCARGGTIDGDYGGRQDFWGQGTMVTVSSFVPVFLPAKPTTTPAPRPPTPAPTIASQPLSLRPEACRPAAGGAVHTRGLDFACDIYIWAPLAGTCGVLLLSLVITLYCNHRNKRGRKKLLYIFKQPFMRPVQTTQEEDGCSCRFPEEEEGGCELRVKFSRSADAPAYQQGQNQLYNELNLGRREEYDVLDKRRGRDPEMGGKPRRKNPQEGLYNELQKDKMAEAYSEIGMKGERRRGKGHDGLYQGLSTATKDTYDALHMQALPPRGSGEGRGSLLTCGDVEENPGPMLLLVTSLLLCELPHPAFLLIPRKVCNGIGIGEFKDSLSINATNIKHFKNCTSISGDLHILPVAFRGDSFTHTPPLDPQELDILKTVKEITGFLLIQAWPENRTDLHAFENLEIIRGRTKQHGQFSLAVVSLNITSLGLRSLKEISDGDVIISGNKNLCYANTINWKKLFGTSGQKTKIISNRGENSCKATGQVCHALCSPEGCWGPEPRDCVSCRNVSRGRECVDKCNLLEGEPREFVENSECIQCHPECLPQAMNITCTGRGPDNCIQCAHYIDGPHCVKTCPAGVMGENNTLVWKYADAGHVCHLCHPNCTYGCTGPGLEGCPTNGPKIPSIATGMVGALLLLLVVALGIGLFM

SEQ ID NO: 52 - DNA, 2667 bp, Artificial Sequence
  FHVH2VH1  CAR nucleic acid sequence
atggccctacctgtgacagccctactgttacccctggccctccttctgcatgctgctagacctcaggtgcagctggtggagtctgggggaggcttggtacagcctggagggtccctgagactctcctgtgcagcctctggattcaccttcagtagttatgaaatgaactgggtccgccaggctccagggaaggggctggagtgggtttcatacattagtagtagtggtagtaccatatactacgcagactctgtgaagggccgattcaccatctccagagacaacgccaagaactcactgtatctgcaaatgaacagtctgagagccgaggacacggctgtttattactgtgcgagagtcgcccagagagaaggggacgtctggggcaaagggaccacggtcaccgtctcctcagggggggggggctctggggggggtggctcaggtggcggtggctctgaagttcagctgctggaaagcggtggtggtctggttcagcctggtggtagcctgcgtctgagctgtgcagcaagcggttttacctttagccatagcgccatgggttgggttcgtcaggcacctggtaaaggtctggaatgggttagcagcatctatgcccgcggcggctatacctattatgcagatagcgttaaaggtcgttttaccattagccgtgataacagcaaaaataccctgtacctgcagatgaatagtctgcgtgcagaggataccgcagtgtattattgtgcgcgcggttaccatctggaatacatggtttctcaggatgtttggggtcaaggtactctggtgaccgtctcctcatttgtgcctgtatttctgcctgccaagcccaccacaacacctgcccctagaccacccacccctgcccccaccattgcttctcagccccttagcttaagacctgaagcctgtagacctgctgctgggggggctgtgcacacaagaggcctggactttgcctgtgacatctacatctgggcccccctggctggcacctgtggggtgctgctgctgagcctggtgatcaccctgtactgcaaccacagaaacaagagaggcagaaagaagctgctgtacatcttcaagcagcccttcatgagacctgtgcagaccacccaagaggaggatggctgcagctgcagattccctgaggaggaggaggggggctgtgagctgagagtgaagttcagcagatctgctgatgcccctgcctatcagcaagggcagaatcagctgtacaatgagctgaatctgggcagaagagaggagtatgatgtgctggacaagagaagaggcagagaccctgagatggggggcaagcctagaagaaagaacccccaagagggcctgtataatgagctgcagaaggacaagatggctgaggcctactctgagattggcatgaagggggagagaagaagaggcaagggccatgatggcctgtaccaaggcctgagcacagccaccaaggacacctatgatgccctacacatgcaagctctgcctcctagaggctctggggaaggaaggggcagcctactgacctgtggggatgtggaggagaaccctggccccatgttgctattagtaaccagcctgctgctgtgtgagctgccccaccctgccttcctgttaatcccacgaaaggtatgtaatggcattggcattggggagtttaaggacagcctgagcatcaatgccaccaacatcaagcacttcaagaactgcacaagcatcagtggggacttgcacatcctgcctgtggccttcagaggggacagcttcacccacaccccccccctggacccccaagagctggacatcctgaagacagtgaaggagatcactggcttcttgctgatccaagcctggcctgagaacagaacagacctgcatgcctttgagaacctggagatcatcagaggcagaaccaagcagcatgggcagttcagcctggctgtggtgagcctgaacatcacaagcctgggcctgagaagcttaaaggagatctctgatggggatgtgatcatctctggcaacaagaacctgtgctatgccaacaccatcaactggaagaagctgtttggcacctctgggcagaagaccaagatcatcagcaacagaggggagaactcctgtaaggccactggccaagtgtgtcatgccctatgcagccctgaggggtgctggggccctgagcctagagactgtgtgagctgcagaaatgtgagcagaggcagagagtgtgtggacaagtgcaacctgctggagggggagcctagagagtttgtggagaactctgagtgtattcagtgtcatcctgagtgcctgccccaagccatgaacatcacctgcactggcagaggccctgacaactgcattcagtgtgcccactacattgatggcccccactgtgtgaagacctgccctgctggggtgatgggggagaacaacaccctggtgtggaagtatgctgatgctggccatgtgtgtcacctgtgccatcccaactgcacctatggctgcactggccctggcctggagggctgccccaccaatggtcccaagattcctagcattgccactggcatggtgggggccctgctcctacttctggtggttgccctgggcattggcctgttcatg

SEQ ID NO: 53 - protein, 889 aa, Artificial Sequence
  FHVH2VH1  CAR protein sequence
MALPVTALLLPLALLLHAARPQVQLVESGGGLVQPGGSLRLSCAASGFTFSSYEMNWVRQAPGKGLEWVSYISSSGSTIYYADSVKGRFTISRDNAKNSLYLQMNSLRAEDTAVYYCARVAQREGDVWGKGTTVTVSSGGGGSGGGGSGGGGSEVQLLESGGGLVQPGGSLRLSCAASGFTFSHSAMGWVRQAPGKGLEWVSSIYARGGYTYYADSVKGRFTISRDNSKNTLYLQMNSLRAEDTAVYYCARGYHLEYMVSQDVWGQGTLVTVSSFVPVFLPAKPTTTPAPRPPTPAPTIASQPLSLRPEACRPAAGGAVHTRGLDFACDIYIWAPLAGTCGVLLLSLVITLYCNHRNKRGRKKLLYIFKQPFMRPVQTTQEEDGCSCRFPEEEEGGCELRVKFSRSADAPAYQQGQNQLYNELNLGRREEYDVLDKRRGRDPEMGGKPRRKNPQEGLYNELQKDKMAEAYSEIGMKGERRRGKGHDGLYQGLSTATKDTYDALHMQALPPRGSGEGRGSLLTCGDVEENPGPMLLLVTSLLLCELPHPAFLLIPRKVCNGIGIGEFKDSLSINATNIKHFKNCTSISGDLHILPVAFRGDSFTHTPPLDPQELDILKTVKEITGFLLIQAWPENRTDLHAFENLEIIRGRTKQHGQFSLAVVSLNITSLGLRSLKEISDGDVIISGNKNLCYANTINWKKLFGTSGQKTKIISNRGENSCKATGQVCHALCSPEGCWGPEPRDCVSCRNVSRGRECVDKCNLLEGEPREFVENSECIQCHPECLPQAMNITCTGRGPDNCIQCAHYIDGPHCVKTCPAGVMGENNTLVWKYADAGHVCHLCHPNCTYGCTGPGLEGCPTNGPKIPSIATGMVGALLLLLVVALGIGLFM

SEQ ID NO: 54 - DNA, 2685 bp, Artificial Sequence
  FHVH4VH1  CAR nucleic acid sequence
atggccctacctgtgacagccctactgttacccctggccctccttctgcatgctgctagacctcaggtccagctggtgcagtctggggctgaggtgaaaaagcccggggagtctctgaggatctcctgtaaggcttctggatacagttttagcaaccattggatcggctgggtgcgccagaagcccgggaaaggcctggagtggatggggagcgtctatcctggtgactccgataccagatacagcccgtccttccaaggccacgtcactgtctcagccgacaagtccatgaataccgcctacctgcagtggagcagcctgaagacctcggacaccgccatgtattattgtgcgagaggtgggactattgacggtgactacggggggaggcaagacttctggggccagggaaccatggtcaccgtctcttcagggggggggggctctggggggggtggctcaggtggcggtggctctgaagttcagctgctggaaagcggtggtggtctggttcagcctggtggtagcctgcgtctgagctgtgcagcaagcggttttacctttagccatagcgccatgggttgggttcgtcaggcacctggtaaaggtctggaatgggttagcagcatctatgcccgcggcggctatacctattatgcagatagcgttaaaggtcgttttaccattagccgtgataacagcaaaaataccctgtacctgcagatgaatagtctgcgtgcagaggataccgcagtgtattattgtgcgcgcggttaccatctggaatacatggtttctcaggatgtttggggtcaaggtactctggtgaccgtctcctcatttgtgcctgtatttctgcctgccaagcccaccacaacacctgcccctagaccacccacccctgcccccaccattgcttctcagccccttagcttaagacctgaagcctgtagacctgctgctgggggggctgtgcacacaagaggcctggactttgcctgtgacatctacatctgggcccccctggctggcacctgtggggtgctgctgctgagcctggtgatcaccctgtactgcaaccacagaaacaagagaggcagaaagaagctgctgtacatcttcaagcagcccttcatgagacctgtgcagaccacccaagaggaggatggctgcagctgcagattccctgaggaggaggaggggggctgtgagctgagagtgaagttcagcagatctgctgatgcccctgcctatcagcaagggcagaatcagctgtacaatgagctgaatctgggcagaagagaggagtatgatgtgctggacaagagaagaggcagagaccctgagatggggggcaagcctagaagaaagaacccccaagagggcctgtataatgagctgcagaaggacaagatggctgaggcctactctgagattggcatgaagggggagagaagaagaggcaagggccatgatggcctgtaccaaggcctgagcacagccaccaaggacacctatgatgccctacacatgcaagctctgcctcctagaggctctggggaaggaaggggcagcctactgacctgtggggatgtggaggagaaccctggccccatgttgctattagtaaccagcctgctgctgtgtgagctgccccaccctgccttcctgttaatcccacgaaaggtatgtaatggcattggcattggggagtttaaggacagcctgagcatcaatgccaccaacatcaagcacttcaagaactgcacaagcatcagtggggacttgcacatcctgcctgtggccttcagaggggacagcttcacccacaccccccccctggacccccaagagctggacatcctgaagacagtgaaggagatcactggcttcttgctgatccaagcctggcctgagaacagaacagacctgcatgcctttgagaacctggagatcatcagaggcagaaccaagcagcatgggcagttcagcctggctgtggtgagcctgaacatcacaagcctgggcctgagaagcttaaaggagatctctgatggggatgtgatcatctctggcaacaagaacctgtgctatgccaacaccatcaactggaagaagctgtttggcacctctgggcagaagaccaagatcatcagcaacagaggggagaactcctgtaaggccactggccaagtgtgtcatgccctatgcagccctgaggggtgctggggccctgagcctagagactgtgtgagctgcagaaatgtgagcagaggcagagagtgtgtggacaagtgcaacctgctggagggggagcctagagagtttgtggagaactctgagtgtattcagtgtcatcctgagtgcctgccccaagccatgaacatcacctgcactggcagaggccctgacaactgcattcagtgtgcccactacattgatggcccccactgtgtgaagacctgccctgctggggtgatgggggagaacaacaccctggtgtggaagtatgctgatgctggccatgtgtgtcacctgtgccatcccaactgcacctatggctgcactggccctggcctggagggctgccccaccaatggtcccaagattcctagcattgccactggcatggtgggggccctgctcctacttctggtggttgccctgggcattggcctgttcatg

SEQ ID NO: 55 - protein, 895 aa, Artificial Sequence
  FHVH4VH1  CAR protein sequence
MALPVTALLLPLALLLHAARPQVQLVQSGAEVKKPGESLRISCKASGYSFSNHWIGWVRQKPGKGLEWMGSVYPGDSDTRYSPSFQGHVTVSADKSMNTAYLQWSSLKTSDTAMYYCARGGTIDGDYGGRQDFWGQGTMVTVSSGGGGSGGGGSGGGGSEVQLLESGGGLVQPGGSLRLSCAASGFTFSHSAMGWVRQAPGKGLEWVSSIYARGGYTYYADSVKGRFTISRDNSKNTLYLQMNSLRAEDTAVYYCARGYHLEYMVSQDVWGQGTLVTVSSFVPVFLPAKPTTTPAPRPPTPAPTIASQPLSLRPEACRPAAGGAVHTRGLDFACDIYIWAPLAGTCGVLLLSLVITLYCNHRNKRGRKKLLYIFKQPFMRPVQTTQEEDGCSCRFPEEEEGGCELRVKFSRSADAPAYQQGQNQLYNELNLGRREEYDVLDKRRGRDPEMGGKPRRKNPQEGLYNELQKDKMAEAYSEIGMKGERRRGKGHDGLYQGLSTATKDTYDALHMQALPPRGSGEGRGSLLTCGDVEENPGPMLLLVTSLLLCELPHPAFLLIPRKVCNGIGIGEFKDSLSINATNIKHFKNCTSISGDLHILPVAFRGDSFTHTPPLDPQELDILKTVKEITGFLLIQAWPENRTDLHAFENLEIIRGRTKQHGQFSLAVVSLNITSLGLRSLKEISDGDVIISGNKNLCYANTINWKKLFGTSGQKTKIISNRGENSCKATGQVCHALCSPEGCWGPEPRDCVSCRNVSRGRECVDKCNLLEGEPREFVENSECIQCHPECLPQAMNITCTGRGPDNCIQCAHYIDGPHCVKTCPAGVMGENNTLVWKYADAGHVCHLCHPNCTYGCTGPGLEGCPTNGPKIPSIATGMVGALLLLLVVALGIGLFM

SEQ ID NO: 56 - DNA, 351 bp, Artificial Sequence
  FHVH2 sdAb nucleic acid sequence
caggtgcagctggtggagtctgggggaggcttggtacagcctggagggtccctgagactctcctgtgcagcctctggattcaccttcagtagttatgaaatgaactgggtccgccaggctccagggaaggggctggagtgggtttcatacattagtagtagtggtagtaccatatactacgcagactctgtgaagggccgattcaccatctccagagacaacgccaagaactcactgtatctgcaaatgaacagtctgagagccgaggacacggctgtttattactgtgcgagagtcgcccagagagaaggggacgtctggggcaaagggaccacggtcaccgtctcctca

SEQ ID NO: 57 - protein, 117 aa, Artificial Sequence
  FHVH2 sdAb protein sequence
QVQLVESGGGLVQPGGSLRLSCAASGFTFSSYEMNWVRQAPGKGLEWVSYISSSGSTIYYADSVKGRFTISRDNAKNSLYLQMNSLRAEDTAVYYCARVAQREGDVWGKGTTVTVSS

SEQ ID NO: 58 - DNA, 369 bp, Artificial Sequence
  FHVH4 sdAb nucleic acid sequence
caggtccagctggtgcagtctggggctgaggtgaaaaagcccggggagtctctgaggatctcctgtaaggcttctggatacagttttagcaaccattggatcggctgggtgcgccagaagcccgggaaaggcctggagtggatggggagcgtctatcctggtgactccgataccagatacagcccgtccttccaaggccacgtcactgtctcagccgacaagtccatgaataccgcctacctgcagtggagcagcctgaagacctcggacaccgccatgtattattgtgcgagaggtgggactattgacggtgactacggggggaggcaagacttctggggccagggaaccatggtcaccgtctcttca

SEQ ID NO: 59 - protein, 123 aa, Artificial Sequence
  FHVH4 sdAb protein sequence
QVQLVQSGAEVKKPGESLRISCKASGYSFSNHWIGWVRQKPGKGLEWMGSVYPGDSDTRYSPSFQGHVTVSADKSMNTAYLQWSSLKTSDTAMYYCARGGTIDGDYGGRQDFWGQGTMVTVSS

SEQ ID NO: 60 - DNA, 759 bp, Artificial Sequence
  FHVH2VH1  sdAb nucleic acid sequence
caggtgcagctggtggagtctgggggaggcttggtacagcctggagggtccctgagactctcctgtgcagcctctggattcaccttcagtagttatgaaatgaactgggtccgccaggctccagggaaggggctggagtgggtttcatacattagtagtagtggtagtaccatatactacgcagactctgtgaagggccgattcaccatctccagagacaacgccaagaactcactgtatctgcaaatgaacagtctgagagccgaggacacggctgtttattactgtgcgagagtcgcccagagagaaggggacgtctggggcaaagggaccacggtcaccgtctcctcagggggggggggctctggggggggtggctcaggtggcggtggctctgaagttcagctgctggaaagcggtggtggtctggttcagcctggtggtagcctgcgtctgagctgtgcagcaagcggttttacctttagccatagcgccatgggttgggttcgtcaggcacctggtaaaggtctggaatgggttagcagcatctatgcccgcggcggctatacctattatgcagatagcgttaaaggtcgttttaccattagccgtgataacagcaaaaataccctgtacctgcagatgaatagtctgcgtgcagaggataccgcagtgtattattgtgcgcgcggttaccatctggaatacatggtttctcaggatgtttggggtcaaggtactctggtgaccgtctcctca

SEQ ID NO: 61 - protein, 253 aa, Artificial Sequence
  FHVH2VH1   sdAb protein sequence
QVQLVESGGGLVQPGGSLRLSCAASGFTFSSYEMNWVRQAPGKGLEWVSYISSSGSTIYYADSVKGRFTISRDNAKNSLYLQMNSLRAEDTAVYYCARVAQREGDVWGKGTTVTVSSGGGGSGGGGSGGGGSEVQLLESGGGLVQPGGSLRLSCAASGFTFSHSAMGWVRQAPGKGLEWVSSIYARGGYTYYADSVKGRFTISRDNSKNTLYLQMNSLRAEDTAVYYCARGYHLEYMVSQDVWGQGTLVTVSS

SEQ ID NO: 62 - DNA, 777 bp, Artificial Sequence
  FHVH4VH1  sdAb nucleic acid sequence
caggtccagctggtgcagtctggggctgaggtgaaaaagcccggggagtctctgaggatctcctgtaaggcttctggatacagttttagcaaccattggatcggctgggtgcgccagaagcccgggaaaggcctggagtggatggggagcgtctatcctggtgactccgataccagatacagcccgtccttccaaggccacgtcactgtctcagccgacaagtccatgaataccgcctacctgcagtggagcagcctgaagacctcggacaccgccatgtattattgtgcgagaggtgggactattgacggtgactacggggggaggcaagacttctggggccagggaaccatggtcaccgtctcttcagggggggggggctctggggggggtggctcaggtggcggtggctctgaagttcagctgctggaaagcggtggtggtctggttcagcctggtggtagcctgcgtctgagctgtgcagcaagcggttttacctttagccatagcgccatgggttgggttcgtcaggcacctggtaaaggtctggaatgggttagcagcatctatgcccgcggcggctatacctattatgcagatagcgttaaaggtcgttttaccattagccgtgataacagcaaaaataccctgtacctgcagatgaatagtctgcgtgcagaggataccgcagtgtattattgtgcgcgcggttaccatctggaatacatggtttctcaggatgtttggggtcaaggtactctggtgaccgtctcctca

SEQ ID NO: 63 - protein, 259 aa, Artificial Sequence
  FHVH4VH1   sdAb protein sequence
QVQLVQSGAEVKKPGESLRISCKASGYSFSNHWIGWVRQKPGKGLEWMGSVYPGDSDTRYSPSFQGHVTVSADKSMNTAYLQWSSLKTSDTAMYYCARGGTIDGDYGGRQDFWGQGTMVTVSSGGGGSGGGGSGGGGSEVQLLESGGGLVQPGGSLRLSCAASGFTFSHSAMGWVRQAPGKGLEWVSSIYARGGYTYYADSVKGRFTISRDNSKNTLYLQMNSLRAEDTAVYYCARGYHLEYMVSQDVWGQGTLVTVSS

SEQ ID NO: 64 - protein, 8 aa, Artificial Sequence
  FHVH2  HCDR1 amino acid sequence
GFTFSSYE

SEQ ID NO: 65 - protein, 8 aa, Artificial Sequence
  FHVH2  HCDR2 amino acid sequence
ISSSGSTI

SEQ ID NO: 66 - protein, 10 aa, Artificial Sequence
  FHVH2  HCDR3 amino acid sequence
ARVAQREGDV

SEQ ID NO: 67 - protein, 8 aa, Artificial Sequence
  FHVH4  HCDR1 amino acid sequence
GYSFSNHW

SEQ ID NO: 68 - protein, 8 aa, Artificial Sequence
  FHVH4  HCDR2 amino acid sequence
VYPGDSDT

SEQ ID NO: 69 - protein, 16 aa, Artificial Sequence
  FHVH4  HCDR3 amino acid sequence
ARGGTIDGDYGGRQDF

SEQ ID NO: 70 - DNA, 20 bp, Artificial Sequence
  CD5 KO sgRNA
gctgtagaactccaccacgc